European Patent Specification EP 4 319 803 B1, published November 26, 2025. Title: CORONAVIRUS VACCINE COMPRISING A MOSAIC PROTEIN. Applicant: VAXTHERA SAS OSORIO, JORGE E. The sequence listing filed with the application follows.

SEQUENCE LISTING (18 sequences)

SEQ ID NO: 1 - protein, 1358 aa, Artificial Sequence
  M-1 (amino acid sequence)
MFLILLISLPTAFAVIGDLNCPLDPRLKGSFNNRDTGPPSISTDTVDVTNGLGTYYVLDRVYLNTTLFLNGYYPTSGSTYRNMALKGTDKLSTLWFKPPFLSDFINGIFAKVKNTKVFKDGVMYSEFPAITIGSTFVNTSYSVVVQPRTINSTQDGVNKLQGLLEVSVCQYNMCEYPHTICHPKLGNHFKELWHLDTGVVSCLYKRNFTYDVNATYLYFHFYQEGGTFYAYFTDTGFVTKFLFNVYLGMALSHYYVMPLTCISRLDIGFTLEYWVTPLTPRQYLLAFNQDGIIFNAVDCMSDFMSEIKCKTQSIAPPTGVYELNGYTVQPIADVYRRKPDLPNCNIEAWLNDKSVPSPLNWERKTFSNCNFNMSSLMSFIQADSFTCNNIDAAKIYGMCFSSITIDKFAIPNRRKVDLQLGNLGYLQSSNYRIDTTATSCQLYYNLPAANVSVSRFNPSTWNKRFGFIEDSVFVPQPTGVFTNHSVVYAQHCFKAPKNFCPCSSCPGKNNGIGTCPAGTNYLTCDNLCTLDPITFKAPDTYKCPQTKSLVGIGEHCSGLAVKSDYCGNNSCTCQPQAFLGWSADSCLQGDKCNIFANFILHDVNNGLTCSTDLQKANTEIELGVCVNYDLYGISGQGIFVEVNATYYNSWQNLLYDSNGNLYGFRDYITNRTFMIHSCYSGRVSAAYHANSSEPALLFRNIKCNYVFNNSLTRQLQPINYSFDSYLGCVVNAYNSTAISVQTCDLTVGSGYCVDYSKNRRSRGAITTGYRFTNFEPFTVNSVNDSLEPVGGLYEIQIPSEFTIGNMEEFIQTSSPKVTIDCAAFVCGDYAACKLQLVEYGSFCDNINAILTEVNELLDTTQLQVANSLMNGVTLSTKLKDGVNFNVDDINFSPVLGCLGSECSKASSRSAIEDLLFDKVKLSDVGFVEAYNNCTGGAEIRDLICVQSYKGIKVLPPLLSENQISGYTLAATSASLFPPWTAAAGVPFYLNVQYRINGLGVTMDVLSQNQKLIANAFNNALHAIQQGFDATNSALVKIQAVVNANAEALNNLLQQLSNRFGAISASLQEILSRLDALEAEAQIDRLINGRLTALNAYVSQQLSDSTLVKFSAAQAMEKVNECVKSQSSRINFCGNGNHIISLVQNAPYGLYFIHFNYVPTKYVTAKVSPGLCIAGNRGIAPKSGYFVNVNNTWMYTGSGYYYPEPITENNVVVMSTCAVNYTKAPYVMLNTSIPNLPDFKEELDQWFKNQTSVAPDLSLDYINVTFLDLQVEMNRLQEAIKVLNHSYINLKDIGTYEYYVKWPWYVWLLICLAGVAMLVLLFFICCCTGCGTSCFKKCGGCCDDYTGYQELVIKTSHDD

SEQ ID NO: 2 - DNA, 4077 bp, Artificial Sequence
  M-1 (nucleic acid sequence)
atgtttttaattttattaatttctttaccaacagcatttgcagtaattggagatttaaattgtccattagatccaagattaaaaggatcttttaataatagagatacaggaccaccatctatttctacagatacagtagatgtaacaaatggattaggaacatattatgtattagatagagtatatttaaatacaacattatttttaaatggatattatccaacatctggatctacatatagaaatatggcattaaaaggaacagataaattatctacattatggtttaaaccaccattcttatctgattttattaatggaatttttgcaaaagtaaaaaatacaaaagtatttaaagatggagtaatgtattctgaatttccagcaattacaattggatctacatttgtaaatacatcttattctgtagtagtacaaccaagaacaattaattctacacaagatggagtaaataaattacaaggattattagaagtatctgtatgtcaatataatatgtgtgaatatccacatacaatttgtcatccaaaattaggaaatcattttaaagaattatggcatttagatacaggagtagtatcttgtttatataaaagaaattttacatatgatgtaaatgcaacatatttatattttcatttctatcaagaaggaggaacattttatgcatattttacagatacaggatttgtaacaaaattcttatttaatgtatatttaggaatggcattatctcattattatgtaatgccattaacatgtatttctagattagatattggatttacattagaatattgggtaacaccattaacaccaagacaatatttattagcatttaatcaagatggaattatttttaatgcagtagattgtatgtctgattttatgtctgaaattaaatgtaaaacacaatctattgcaccaccaacaggagtatatgaattaaatggatatacagtacaaccaattgcagatgtatatagaagaaaaccagatttaccaaattgtaatattgaagcatggttaaatgataaatctgtaccatctccattaaattgggaaagaaaaacattttctaattgtaattttaatatgtcttctttaatgtcttttattcaagcagattcttttacatgtaataatattgatgcagcaaaaatttatggaatgtgtttctcttctattacaattgataaatttgcaattccaaatagaagaaaagtagatttacaattaggaaatttaggatatttacaatcttctaattatagaattgatacaacagcaacatcttgtcaattatattataatttaccagcagcaaatgtatctgtatctagatttaatccatctacatggaataaaagatttggatttattgaagattctgtatttgtaccacaaccaacaggagtatttacaaatcattctgtagtatatgcacaacattgttttaaagcaccaaaaaatttctgtccatgttcttcttgtccaggaaaaaataatggaattggaacatgtccagcaggaacaaattatttaacatgtgataatttatgtacattagatccaattacatttaaagcaccagatacatataaatgtccacaaacaaaatctttagtaggaattggagaacattgttctggattagcagtaaaatctgattattgtggaaataattcttgtacatgtcaaccacaagcatttttaggatggtctgcagattcttgtttacaaggagataaatgtaatatttttgcaaattttattttacatgatgtaaataatggattaacatgttctacagatttacaaaaagcaaatacagaaattgaattaggagtatgtgtaaattatgatttatatggaatttctggacaaggaattttcgtagaagtaaatgcaacatattataattcttggcaaaatttattatatgattctaatggaaatttatatggatttagagattatattacaaatagaacatttatgattcattcttgttattctggaagagtatctgcagcatatcatgcaaattcttctgaaccagcattattatttagaaatattaaatgtaattatgtatttaataattctttaacaagacaattacaaccaattaattattcttttgattcttatttaggatgtgtagtaaatgcatataattctacagcaatttctgtacaaacatgtgatttaacagtaggatctggatattgtgtagattattctaaaaatagaagatctagaggagcaattacaacaggatatagatttacaaattttgaaccatttacagtaaattctgtaaatgattctttagaaccagtaggaggattatatgaaattcaaattccatctgaatttacaattggaaatatggaagaatttattcaaacatcttctccaaaagtaacaattgattgtgcagcatttgtatgtggagattatgcagcatgtaaattacaattagtagaatatggatctttctgtgataatattaatgcaattttaacagaagtaaatgaattattagatacaacacaattacaagtagcaaattctttaatgaatggagtaacattatctacaaaattaaaagatggagtaaattttaatgtagatgatattaatttctctccagtattaggatgtttaggatctgaatgttctaaagcatcttctagatctgcaattgaagatttattatttgataaagtaaaattatctgatgtaggatttgtagaagcatataataattgtacaggaggagcagaaattagagatttaatttgtgtacaatcttataaaggaattaaagtattaccaccattattatctgaaaatcaaatttctggatatacattagcagcaacatctgcatctttatttccaccatggacagcagcagcaggagtaccattttatttaaatgtacaatatagaattaatggattaggagtaacaatggatgtattatctcaaaatcaaaaattaattgcaaatgcatttaataatgcattacatgcaattcaacaaggatttgatgcaacaaattctgcattagtaaaaattcaagcagtagtaaatgcaaatgcagaagcattaaataatttattacaacaattatctaatagatttggagcaatttctgcatctttacaagaaattttatctagattagatgcattagaagcagaagcacaaattgatagattaattaatggaagattaacagcattaaatgcatatgtatctcaacaattatctgattctacattagtaaaattttctgcagcacaagcaatggaaaaagtaaatgaatgtgtaaaatctcaatcttctagaattaatttctgtggaaatggaaatcatattatttctttagtacaaaatgcaccatatggattatattttattcattttaattatgtaccaacaaaatatgtaacagcaaaagtatctccaggattatgtattgcaggaaatagaggaattgcaccaaaatctggatattttgtaaatgtaaataatacatggatgtatacaggatctggatattattatccagaaccaattacagaaaataatgtagtagtaatgtctacatgtgcagtaaattatacaaaagcaccatatgtaatgttaaatacatctattccaaatttaccagattttaaagaagaattagatcaatggtttaaaaatcaaacatctgtagcaccagatttatctttagattatattaatgtaacatttttagatttacaagtagaaatgaatagattacaagaagcaattaaagtattaaatcattcttatattaatttaaaagatattggaacatatgaatattatgtaaaatggccatggtatgtatggttattaatttgtttagcaggagtagcaatgttagtattattatttttcatttgttgttgtacaggatgtggaacatcttgttttaaaaaatgtggaggatgttgtgatgattatacaggatatcaagaattagtaattaaaacatctcatgatgattaa

SEQ ID NO: 3 - protein, 1353 aa, Artificial Sequence
  M-2 (amino acid sequence)
MIHSVFLLMFLLTPTESYVDVGPDSVKSACIEVDIQQTFFDKTWPRPIDVSKADGIIYPQGRTYSNITITYQGLFPYQGDHGDMYVYSAGHATGTTPQKLFVANYSQDVKQFANGFVVRIGAAANSTGTVIISPSTSATIRKIYPAFMLGSSVGNFSDGKMGRFFNHTLVLLPDGCGTLLRAFYCILEPRSGNHCPAGNSYTSFATYHTPATDCSDGNYNRNASLNSFKEYFNLRNCTFMYTYNITEDEILEWFGITQTAQGVHLFSSRYVDLYGGNMFQFATLPVYDTIKYYSIIPHSIRSIQSDRKAWAAFYVYKLQPLTFLLDFSVDGYIRRAIDCGFNDLSQLHCSYESFDVESGVYSVSSFEAKPSGSVVEQAEGVECDFSPLLSGTPPQVYNFKRLVFTNCNYNLTKLLSLFSVNDFTCSQISPAAIASNCYSSLILDYFSYPLSMKSDLSVSSAGPISQFNYKQSFSNPTCLILATVPHNLTTITKPLKYSYINKCSRLLSDDRTEVPQLVNANQYSPCVSIVPSTVWEDGDYYRKQLSPLEGGGWLVASGSTVAMTEQLQMGFGITVQYGTDTNSVCPKLEFANDTKIASQLGNCVEYSLYGVSGRGVFQNCTAVGVRQQRFVYDAYQNLVGYYSDDGNYYCLRACVSVPVSVIYDKETKTHATLFGSVACEHISSTMSQYSRSTRSMLKRRDSTYGPLQTPVGCVLGLVNSSLFVEDCKLPLGQSLCALPDTPSTLTPRSVRSVPGEMRLASIAFNHPIQVDQLNSSYFKLSIPTNFSFGVTQEYIQTTIQKVTVDCKQYVCNGFQKCEQLLREYGQFCSKINQALHGANLRQDDSVRNLFASVKSSQSSPIIPGFGGDFNLTLLEPVSISTGSRSARSAIEDLLFDKVTIADPGYMQGYDDCMQQGPASARDLICAQYVAGYKVLPPLMDVNMEAAYTSSLLGSIAGVGWTAGLSSFAAIPFAQSIFYRLNGVGITQQVLSENQKLIANKFNQALGAMQTGFTTTNEAFRKVQDAVNNNAQALSKLASELSNTFGAISASIGDIIQRLDVLEQDAQIDRLINGRLTTLNAFVAQQLVRSESAALSAQLAKDKVNECVKAQSKRSGFCGQGTHIVSFVVNAPNGLYFMHVGYYPSNHIEVVSAYGLCDAANPTNCIAPVNGYFIKTNNTRIVDEWSYTGSSFYAPEPITSLNTKYVAPQVTYQNISTNLPPPLLGNSTGIDFQDELDEFFKNVSTSIPNFGSLTQINTTLLDLTYEMLSLQQVVKALNESYIDLKELGNYTYYNKWPWYIWLGFIAGLVALALCVFFILCCTGCGTNCMGKLKCNRCCDRYEEYDLEPHKVHVH

SEQ ID NO: 4 - DNA, 4062 bp, Artificial Sequence
  M-2 (nucleic acid sequence)
atgattcattctgttttcttattaatgttcttattaacaccaacagaatcttatgtagatgtaggaccagattctgtaaaatctgcatgtattgaagtagatattcaacaaacattttttgataaaacatggccaagaccaattgatgtatctaaagcagatggaattatttatccacaaggaagaacatattctaatattacaattacatatcaaggattatttccatatcaaggagatcatggagatatgtatgtatattctgcaggacatgcaacaggaacaacaccacaaaaattatttgtagcaaattattctcaagatgtaaaacaatttgcaaatggatttgtagtaagaattggagcagcagcaaattctacaggaacagtaattatttctccatctacatctgcaacaattagaaaaatttatccagcatttatgttaggatcttctgtaggaaatttctctgatggaaaaatgggaagattttttaatcatacattagtattattaccagatggatgtggaacattattaagagcattttattgtattttagaaccaagatctggaaatcattgtccagcaggaaattcttatacatcttttgcaacatatcatacaccagcaacagattgttctgatggaaattataatagaaatgcatctttaaattcttttaaagaatattttaatttaagaaattgtacatttatgtatacatataatattacagaagatgaaattttagaatggtttggaattacacaaacagcacaaggagtacatttattttcttctagatatgtagatttatatggaggaaatatgtttcaatttgcaacattaccagtatatgatacaattaaatattattctattattccacattctattagatctattcaatctgatagaaaagcatgggcagcattttatgtatataaattacaaccattaactttcttattagatttctctgtagatggatatattagaagagcaattgattgtggatttaatgatttatctcaattacattgttcttatgaatcttttgatgtagaatctggagtatattctgtatcttcttttgaagcaaaaccatctggatctgtagtagaacaagcagaaggagtagaatgtgatttctctccattattatctggaacaccaccacaagtatataattttaaaagattagtatttacaaattgtaattataatttaacaaaattattatctttattttctgtaaatgattttacatgttctcaaatttctccagcagcaattgcatctaattgttattcttctttaattttagattatttctcttatccattatctatgaaatctgatttatctgtatcttctgcaggaccaatttctcaatttaattataaacaatctttctctaatccaacatgtttaattttagcaacagtaccacataatttaacaacaattacaaaaccattaaaatattcttatattaataaatgttctagattattatctgatgatagaacagaagtaccacaattagtaaatgcaaatcaatattctccatgtgtatctattgtaccatctacagtatgggaagatggagattattatagaaaacaattatctccattagaaggaggaggatggttagtagcatctggatctacagtagcaatgacagaacaattacaaatgggatttggaattacagtacaatatggaacagatacaaattctgtatgtccaaaattagaatttgcaaatgatacaaaaattgcatctcaattaggaaattgtgtagaatattctttatatggagtatctggaagaggagtatttcaaaattgtacagcagtaggagtaagacaacaaagatttgtatatgatgcatatcaaaatttagtaggatattattctgatgatggaaattattattgtttaagagcatgtgtatctgtaccagtatctgtaatttatgataaagaaacaaaaacacatgcaacattatttggatctgtagcatgtgaacatatttcttctacaatgtctcaatattctagatctacaagatctatgttaaaaagaagagattctacatatggaccattacaaacaccagtaggatgtgtattaggattagtaaattcttctttatttgtagaagattgtaaattaccattaggacaatctttatgtgcattaccagatacaccatctacattaacaccaagatctgtaagatctgtaccaggagaaatgagattagcatctattgcatttaatcatccaattcaagtagatcaattaaattcttcttattttaaattatctattccaacaaatttctcttttggagtaacacaagaatatattcaaacaacaattcaaaaagtaacagtagattgtaaacaatatgtatgtaatggatttcaaaaatgtgaacaattattaagagaatatggacaattttgttctaaaattaatcaagcattacatggagcaaatttaagacaagatgattctgtaagaaatttatttgcatctgtaaaatcttctcaatcttctccaattattccaggatttggaggagattttaatttaacattattagaaccagtatctatttctacaggatctagatctgcaagatctgcaattgaagatttattatttgataaagtaacaattgcagatccaggatatatgcaaggatatgatgattgtatgcaacaaggaccagcatctgcaagagatttaatttgtgcacaatatgtagcaggatataaagtattaccaccattaatggatgtaaatatggaagcagcatatacatcttctttattaggatctattgcaggagtaggatggacagcaggattatcttcttttgcagcaattccatttgcacaatctatattctatagattaaatggagtaggaattacacaacaagtattatctgaaaatcaaaaattaattgcaaataaatttaatcaagcattaggagcaatgcaaacaggatttacaacaacaaatgaagcatttagaaaagtacaagatgcagtaaataataatgcacaagcattatctaaattagcatctgaattatctaatacatttggagcaatttctgcatctattggagatattattcaaagattagatgtattagaacaagatgcacaaattgatagattaattaatggaagattaacaacattaaatgcatttgtagcacaacaattagtaagatctgaatctgcagcattatctgcacaattagcaaaagataaagtaaatgaatgtgtaaaagcacaatctaaaagatctggattttgtggacaaggaacacatattgtatcttttgtagtaaatgcaccaaatggattatattttatgcatgtaggatattatccatctaatcatattgaagtagtatctgcatatggattatgtgatgcagcaaatccaacaaattgtattgcaccagtaaatggatattttattaaaacaaataatacaagaattgtagatgaatggtcttatacaggatcttctttctatgcaccagaaccaattacatctttaaatacaaaatatgtagcaccacaagtaacatatcaaaatatttctacaaatttaccaccaccattattaggaaattctacaggaattgattttcaagatgaattagatgaattttttaaaaatgtatctacatctattccaaattttggatctttaacacaaattaatacaacattattagatttaacatatgaaatgttatctttacaacaagtagtaaaagcattaaatgaatcttatattgatttaaaagaattaggaaattatacatattataataaatggccatggtatatttggttaggatttattgcaggattagtagcattagcattatgtgtattctttattttatgttgtacaggatgtggaacaaattgtatgggaaaattaaaatgtaatagatgttgtgatagatatgaagaatatgatttagaaccacataaagtacatgtacattaa

SEQ ID NO: 5 - protein, 1356 aa, Artificial Sequence
  M-3 (amino acid sequence)
MKLFLILLVLPLASCFFTCNSNANLSMLQLGVPDNSSTIVTGLLPTHWICANQSTSVYSANGFFYIDVGNHRSAFALHTGYYDVNQYYIYVTNEIGLNASVTLKICKFGINTTFDFLSNSSSSFDCIVNLLFTEQLGAPLGITISGETVRLHLYNVTRTFYVPAAYKLTKLSVKCYFNYSCVFSVVNATVTVNVTTHNGRVVNYTVCDDCNGYTDNIFSVQQDGRIPNGFPFNNWFLLTNGSTLVDGVSRLYQPLRLTCLWPVPGLKSSTGFVYFNATGSDVNCNGYQHNSVADVMRYNLNFSANSVDNLKSGVIVFKTLQYDVLFYCSNSSSGVLDTTIPFGPSSQPYYCFINSTINTTHVSTFVGVLPPTVREIVVARTGQFYINGFKYFDLGFIEAVNFNVTTASATDFWTVAFATFVDVLVNVSATKIQNLLYCDSPFEKLQCEHLQFGLQDGFYSANFLDDNVLPETYVALPIYYQHTDINFTATASFGGSCYVCKPHQVNISLNGNTSVCVRTSHFSIRYIYNRVKSGSPGDSSWHIYLKSGTCPFSFSKLNNFQKFKTICFSTVAVPGSCNFPLEATWHYTSYTIVGALYVTWSEGNSITGVPYPVSGIREFSNLVLNNCTKYNIYDYVGTGIIRSSNQSLAGGITYVSNSGNLLGFKNVSTGNIFIVTPCNQPDQVAVYQQSIIGAMTAVNESRYGLQNLLQLPNFYYVSNGGNNCTTAVMTYSNFGICADGSLIPVRPRNSSDNGISAIITANLSIPSNWTTSVQVEYLQITSTPIVVDCATYVCNGNPRCKNLLKQYTSACKTIEDALRLSAHLETNDVSSMLTFDSNAFSLANVTSFGDYNLSSVLPQRNIHSSRIAGRSALEDLLFSKVVTSGLGTVDVDYKSCTKGLSIADLACAQYYNGIMVLPGVADAERMAMYTGSLIGGMVLGGLTSAAAIPFSLALQARLNYVALQTDVLQENQKILAASFNKAINNIVASFSSVNDAITQTAEAIHTVTIALNKIQDVVNQQGSALNHLTSQLRHNFQAISNSIQAIYDRLDSIQADQQVDRLITGRLAALNAFVSQVLNKYTEVRSSRRLAQQKINECVKSQSNRYGFCGNGTHIFSIVNSAPDGLLFLHTVLLPTDYKNVKAWSGICVDGIYGYVLRQPNLVLYSDNGVFRVTSRVMFQPRLPVLSDFVQIYNCNVTFVNISRVELHTVIPDYVDVNKTLQEFAQNLPKYVKPNFDLTPFNLTYLNLSSELKQLEAKTASLFQTTVELQGLIDQINSTYVDLKLLNRFENYIKWPWWVWLIISVVFVVLLSLLVFCCLSTGCCGCCNCLTSSMRGCCDCGSTKLPYYEFEKVHVQ

SEQ ID NO: 6 - DNA, 4071 bp, Artificial Sequence
  M-3 (nucleic acid sequence)
atgaaattatttttaattttattagtattaccattagcatcttgtttttttacatgtaattctaatgcaaatttatctatgttacaattaggagtaccagataattcttctacaattgtaacaggattattaccaacacattggatttgtgcaaatcaatctacatctgtatattctgcaaatggattcttctatattgatgtaggaaatcatagatctgcatttgcattacatacaggatattatgatgtaaatcaatattatatttatgtaacaaatgaaattggattaaatgcatctgtaacattaaaaatttgtaaatttggaattaatacaacatttgatttcttatctaattcttcttcttcttttgattgtattgtaaatttattatttacagaacaattaggagcaccattaggaattacaatttctggagaaacagtaagattacatttatataatgtaacaagaacattttatgtaccagcagcatataaattaacaaaattatctgtaaaatgttattttaattattcttgtgtattttctgtagtaaatgcaacagtaacagtaaatgtaacaacacataatggaagagtagtaaattatacagtatgtgatgattgtaatggatatacagataatattttctctgtacaacaagatggaagaattccaaatggatttccatttaataattggttcttattaacaaatggatctacattagtagatggagtatctagattatatcaaccattaagattaacatgtttatggccagtaccaggattaaaatcttctacaggatttgtatattttaatgcaacaggatctgatgtaaattgtaatggatatcaacataattctgtagcagatgtaatgagatataatttaaatttctctgcaaattctgtagataatttaaaatctggagtaattgtatttaaaacattacaatatgatgtattattttattgttctaattcttcttctggagtattagatacaacaattccatttggaccatcttctcaaccatattattgttttattaattctacaattaatacaacacatgtatctacatttgtaggagtattaccaccaacagtaagagaaattgtagtagcaagaacaggacaattttatattaatggatttaaatattttgatttaggatttattgaagcagtaaattttaatgtaacaacagcatctgcaacagatttttggacagtagcatttgcaacatttgtagatgtattagtaaatgtatctgcaacaaaaattcaaaatttattatattgtgattctccatttgaaaaattacaatgtgaacatttacaatttggattacaagatggattttattctgcaaattttttagatgataatgtattaccagaaacatatgtagcattaccaatttattatcaacatacagatattaattttacagcaacagcatcttttggaggatcttgttatgtatgtaaaccacatcaagtaaatatttctttaaatggaaatacatctgtatgtgtaagaacatctcatttctctattagatatatttataatagagtaaaatctggatctccaggagattcttcttggcatatttatttaaaatctggaacatgtccattttctttctctaaattaaataattttcaaaaatttaaaacaatttgtttctctacagtagcagtaccaggatcttgtaattttccattagaagcaacatggcattatacatcttatacaattgtaggagcattatatgtaacatggtctgaaggaaattctattacaggagtaccatatccagtatctggaattagagaattttctaatttagtattaaataattgtacaaaatataatatttatgattatgtaggaacaggaattattagatcttctaatcaatctttagcaggaggaattacatatgtatctaattctggaaatttattaggatttaaaaatgtatctacaggaaatatattcattgtaacaccatgtaatcaaccagatcaagtagcagtatatcaacaatctattattggagcaatgacagcagtaaatgaatctagatatggattacaaaatttattacaattaccaaacttctattatgtatctaatggaggaaataattgtacaacagcagtaatgacatattctaattttggaatttgtgcagatggatctttaattccagtaagaccaagaaattcttctgataatggaatttctgcaattattacagcaaatttatctattccatctaattggacaacatctgtacaagtagaatatttacaaattacatctacaccaattgtagtagattgtgcaacatatgtatgtaatggaaatccaagatgtaaaaatttattaaaacaatatacatctgcatgtaaaacaattgaagatgcattaagattatctgcacatttagaaacaaatgatgtatcttctatgttaacatttgattctaatgcattttctttagcaaatgtaacatcttttggagattataatttatcttctgtattaccacaaagaaatattcattcttctagaattgcaggaagatctgcattagaagatttattattttctaaagtagtaacatctggattaggaacagtagatgtagattataaatcttgtacaaaaggattatctattgcagatttagcatgtgcacaatattataatggaattatggtattaccaggagtagcagatgcagaaagaatggcaatgtatacaggatctttaattggaggaatggtattaggaggattaacatctgcagcagcaattccattttctttagcattacaagcaagattaaattatgtagcattacaaacagatgtattacaagaaaatcaaaaaattttagcagcatcttttaataaagcaattaataatattgtagcatctttctcttctgtaaatgatgcaattacacaaacagcagaagcaattcatacagtaacaattgcattaaataaaattcaagatgtagtaaatcaacaaggatctgcattaaatcatttaacatctcaattaagacataattttcaagcaatttctaattctattcaagcaatttatgatagattagattctattcaagcagatcaacaagtagatagattaattacaggaagattagcagcattaaatgcatttgtatctcaagtattaaataaatatacagaagtaagatcttctagaagattagcacaacaaaaaattaatgaatgtgtaaaatctcaatctaatagatatggattttgtggaaatggaacacatattttctctattgtaaattctgcaccagatggattattatttttacatacagtattattaccaacagattataagaatgtaaaagcatggtctggaatttgtgtagatggaatttatggatatgtattaagacaaccaaatttagtattatattctgataatggagtatttagagtaacatctagagtaatgtttcaaccaagattaccagtattatctgattttgtacaaatttataattgtaatgtaacatttgtaaatatttctagagtagaattacatacagtaattccagattatgtagatgtaaataaaacattacaagaatttgcacaaaatttaccaaaatatgtaaaaccaaattttgatttaacaccatttaatttaacatatttaaatttatcttctgaattaaaacaattagaagcaaaaacagcatctttatttcaaacaacagtagaattacaaggattaattgatcaaattaattctacatatgtagatttaaaattattaaatagatttgaaaattatattaaatggccatggtgggtatggttaattatttctgtagtatttgtagtattattatctttattagtattttgttgtttatctacaggatgttgtggatgttgtaattgtttaacatcttctatgagaggatgttgtgattgtggatctacaaaattaccatattatgaatttgaaaaagtacatgtacaataa

SEQ ID NO: 7 - DNA, 42 bp, Artificial Sequence
  S E/L Promoter (nucleic acid sequence)
aaaaattgaaattttattttttttttttggaatataaataag

SEQ ID NO: 8 - DNA, 88 bp, Artificial Sequence
  LEO Promoter (nucleic acid sequence)
ttttattttttttttttggaatataaatatccggtaaaattgaaaaaatatacactaattagcgtctcgtttcagacgctagctcgag

SEQ ID NO: 9 - protein, 1270 aa, Artificial Sequence
  M-4 (amino acid sequence)
MFVFLVLLPLVSSQCVNLTTRTQLPPAYTNSFTRGVYYPDKVFRSSVLHSTQDLFLPFFSNVTWFHAIHVSGTNGTKRFDNPVLPFNDGVYFASTEKSNIIRGWIFGTTLDSKTQSLLIVNNATNVVIKVCEFQFCNYPFLYHKNNKSWMESEFRVYSSANNCTFEYVSQPFLMDLEGKHGNFKNLREFVFKNIDGYFKIYSKHTPINLVRDLPQGFSALEPLVDLPIGINITRFQTLLALHRSYLTPGDSSSGWTAGAAAYYVGYLQPRTFLLKYNENGTITDAVDCALDPLSETKCTLKSFTVEKGIYQTSNFRVQPTESIVRFPNITNLCPFGEVFNATRFASVYAWNRKRISNCVADYSVLYNSASFSTFKCYGVSPTKLNDLCFTNVYADSFVIRGDEVRQIAPGQTGTIADYNYKLPDDFTGCVIAWNSNNLDSKVGGNYNYLYRLFRKSNLKPFERDISTEIYQAGSKPCNGVKGFNCYFPLQPYGFQPTYGVGYQPYRVVVLSFELLHAPATVCGPKKSTNLVKNKCVNFNFNGLTGTGVLTESNKKFLPFQQFGRDIADTTDAVRDPQTLEILDITPCSFGGVSVITPGTNTSNQVAVLYQGVNCTEVPVAIHADQLTPTWRVYSTGSNVFQTRAGCLIGAEHVNNSYECDIPIGAGICASYQTQTNSPRRARSVASQSIIAYTMSLGAENSVAYSNNSIAIPTNFTISVTTEILPVSMTKTSVDCTMYICGDSTECSNLLLQYGSFCTQLNRALTGIAVEQDKNTQEVFAQVKQIYKTPPIKDFGGFNFSQILPDPSKPSKRSFIEDLLFNKVTLADAGFIKQYGDCLGDIAARDLICAQKFNGLTVLPPLLTDEMVAQYTSALLAGTITSGWTFGAGAALQIPFAMQMAYRFNGIGVTQNVLYENQKLIANQFNSAIGKIQDSLSSTASALGKLQDVVNQNAQALNTLVKQLSSNFGAISSVLNDILSRLDKVEAEVQIDRLITGRLQSLQTYVTQQLIRAAEIRASANLAATKMSECVLGQSKRVDFCGKGYHLMSFPQSAPHGVVFLHVTYVPAQEKNFTTAPAICHDGKAHFPREGVFVSNGTHWFVTQRNFYEPQIITTDNTFVSGNCDVVIGIVNNTVYDPLQPELDSFKEELDKYFKNHTSPDVDLGDISGINASFVNIQKEIDRLNEVAKNLNESLIDLQELGKYEQYIKWPWYIWLGFIAGLIAIVMVTIMLCCMTSCCSCLKGCCSCGSCCKFDEDDSEPVLKGVKLHYT

SEQ ID NO: 10 - DNA, 3813 bp, Artificial Sequence
  M-4 (nucleic acid sequence)
atgtttgtatttttagtattattaccattagtatcttctcaatgtgtaaatttaactactagaactcaattaccaccagcttatactaattcttttactagaggagtatattatccagataaagtatttagatcttctgtattacattctactcaagatttatttttaccattcttctctaatgtaacttggtttcatgctattcatgtatctggaactaatggaactaaaagatttgataatccagtattaccatttaatgatggagtatattttgcttctactgaaaaatctaatattattagaggatggatttttggaactactttagattctaaaactcaatctttattaattgtaaataatgctactaatgtagtaattaaagtatgtgaatttcaattttgtaattatccattcttatatcataaaaataataaatcttggatggaatctgaatttagagtatattcttctgctaataattgtacttttgaatatgtatctcaaccatttttaatggatttagaaggaaaacatggaaattttaaaaatttaagagaatttgtatttaaaaatattgatggatattttaaaatttattctaaacatactccaattaatttagtaagagatttaccacaaggattttctgctttagaaccattagtagatttaccaattggaattaatattactagatttcaaactttattagctttacatagatcttatttaactccaggagattcttcttctggatggactgctggagctgctgcttattatgtaggatatttacaaccaagaactttcttattaaaatataatgaaaatggaactattactgatgctgtagattgtgctttagatccattatctgaaactaaatgtactttaaaatcttttactgtagaaaaaggaatttatcaaacttctaattttagagtacaaccaactgaatctattgtaagatttccaaatattactaatttatgtccatttggagaagtatttaatgctactagatttgcttctgtatatgcttggaatagaaaaagaatttctaattgtgtagctgattattctgtattatataattctgcttctttctctacttttaaatgttatggagtatctccaactaaattaaatgatttatgttttactaatgtatatgctgattcttttgtaattagaggagatgaagtaagacaaattgctccaggacaaactggaactattgctgattataattataaattaccagatgattttactggatgtgtaattgcttggaattctaataatttagattctaaagtaggaggaaattataattatttatatagattatttagaaaatctaatttaaaaccatttgaaagagatatttctactgaaatttatcaagctggatctaaaccatgtaatggagtaaaaggatttaattgttattttccattacaaccatatggatttcaaccaacttatggagtaggatatcaaccatatagagtagtagtattatcttttgaattattacatgctccagctactgtatgtggaccaaaaaaatctactaatttagtaaaaaataaatgtgtaaattttaattttaatggattaactggaactggagtattaactgaatctaataaaaaatttttaccatttcaacaatttggaagagatattgctgatactactgatgctgtaagagatccacaaactttagaaattttagatattactccatgttcttttggaggagtatctgtaattactccaggaactaatacttctaatcaagtagctgtattatatcaaggagtaaattgtactgaagtaccagtagctattcatgctgatcaattaactccaacttggagagtatattctactggatctaatgtatttcaaactagagctggatgtttaattggagctgaacatgtaaataattcttatgaatgtgatattccaattggagctggaatttgtgcttcttatcaaactcaaactaattctccaagaagagctagatctgtagcttctcaatctattattgcttatactatgtctttaggagctgaaaattctgtagcttattctaataattctattgctattccaactaattttactatttctgtaactactgaaattttaccagtatctatgactaaaacttctgtagattgtactatgtatatttgtggagattctactgaatgttctaatttattattacaatatggatctttttgtactcaattaaatagagctttaactggaattgctgtagaacaagataaaaatactcaagaagtatttgctcaagtaaaacaaatttataaaactccaccaattaaagattttggaggatttaatttctctcaaattttaccagatccatctaaaccatctaaaagatcttttattgaagatttattatttaataaagtaactttagctgatgctggatttattaaacaatatggagattgtttaggagatattgctgctagagatttaatttgtgctcaaaaatttaatggattaactgtattaccaccattattaactgatgaaatggtagctcaatatacttctgctttattagctggaactattacttctggatggacttttggagctggagctgctttacaaattccatttgctatgcaaatggcttatagatttaatggaattggagtaactcaaaatgtattatatgaaaatcaaaaattaattgctaatcaatttaattctgctattggaaaaattcaagattctttatcttctactgcttctgctttaggaaaattacaagatgtagtaaatcaaaatgctcaagctttaaatactttagtaaaacaattatcttctaattttggagctatttcttctgtattaaatgatattttatctagattagataaagtagaagctgaagtacaaattgatagattaattactggaagattacaatctttacaaacttatgtaactcaacaattaattagagctgctgaaattagagcttctgctaatttagctgctactaaaatgtctgaatgtgtattaggacaatctaaaagagtagatttttgtggaaaaggatatcatttaatgtcttttccacaatctgctccacatggagtagtatttttacatgtaacttatgtaccagctcaagaaaaaaattttactactgctccagctatttgtcatgatggaaaagctcattttccaagagaaggagtatttgtatctaatggaactcattggtttgtaactcaaagaaatttctatgaaccacaaattattactactgataatacttttgtatctggaaattgtgatgtagtaattggaattgtaaataatactgtatatgatccattacaaccagaattagattcttttaaagaagaattagataaatattttaaaaatcatacttctccagatgtagatttaggagatatttctggaattaatgcttcttttgtaaatattcaaaaagaaattgatagattaaatgaagtagctaaaaatttaaatgaatctttaattgatttacaagaattaggaaaatatgaacaatatattaaatggccatggtatatttggttaggatttattgctggattaattgctattgtaatggtaactattatgttatgttgtatgacttcttgttgttcttgtttaaaaggatgttgttcttgtggatcttgttgtaaatttgatgaagatgattctgaaccagtattaaaaggagtaaaattacattatacttaa

SEQ ID NO: 11 - protein, 1273 aa, Artificial Sequence
  M-B (amino acid sequence)
MFVFLVLLPLVSSQCVNLTTRTQLPPAYTNSFTRGVYYPDKVFRSSVLHSTQDLFLPFFSNVTWFHAIHVSGTNGTKRFDNPVLPFNDGVYFASTEKSNIIRGWIFGTTLDSKTQSLLIVNNATNVVIKVCEFQFCNDPFLGVYYHKNNKSWMESEFRVYSSANNCTFEYVSQPFLMDLEGKQGNFKNLREFVFKNIDGYFKIYSKHTPINLVRDLPQGFSALEPLVDLPIGINITRFQTLLALHRSYLTPGDSSSGWTAGAAAYYVGYLQPRTFLLKYNENGTITDAVDCALDPLSETKCTLKSFTVEKGIYQTSNFRVQPTESIVRFPNITNLCPFGEVFNATRFASVYAWNRKRISNCVADYSVLYNSASFSTFKCYGVSPTKLNDLCFTNVYADSFVIRGDEVRQIAPGQTGKIADYNYKLPDDFTGCVIAWNSNNLDSKVGGNYNYLYRLFRKSNLKPFERDISTEIYQAGSTPCNGVEGFNCYFPLQSYGFQPTNGVGYQPYRVVVLSFELLHAPATVCGPKKSTNLVKNKCVNFNFNGLTGTGVLTESNKKFLPFQQFGRDIADTTDAVRDPQTLEILDITPCSFGGVSVITPGTNTSNQVAVLYQGVNCTEVPVAIHADQLTPTWRVYSTGSNVFQTRAGCLIGAEHVNNSYECDIPIGAGICASYQTQTNSPRRARSVASQSIIAYTMSLGAENSVAYSNNSIAIPTNFTISVTTEILPVSMTKTSVDCTMYICGDSTECSNLLLQYGSFCTQLNRALTGIAVEQDKNTQEVFAQVKQIYKTPPIKDFGGFNFSQILPDPSKPSKRSFIEDLLFNKVTLADAGFIKQYGDCLGDIAARDLICAQKFNGLTVLPPLLTDEMIAQYTSALLAGTITSGWTFGAGAALQIPFAMQMAYRFNGIGVTQNVLYENQKLIANQFNSAIGKIQDSLSSTASALGKLQDVVNQNAQALNTLVKQLSSNFGAISSVLNDILSRLDKVEAEVQIDRLITGRLQSLQTYVTQQLIRAAEIRASANLAATKMSECVLGQSKRVDFCGKGYHLMSFPQSAPHGVVFLHVTYVPAQEKNFTTAPAICHDGKAHFPREGVFVSNGTHWFVTQRNFYEPQIITTDNTFVSGNCDVVIGIVNNTVYDPLQPELDSFKEELDKYFKNHTSPDVDLGDISGINASVVNIQKEIDRLNEVAKNLNESLIDLQELGKYEQYIKWPWYIWLGFIAGLIAIVMVTIMLCCMTSCCSCLKGCCSCGSCCKFDEDDSEPVLKGVKLHYT

SEQ ID NO: 12 - DNA, 3822 bp, Artificial Sequence
  M-B (nucleic acid sequence)
atgtttgtatttttagtattattaccattagtatcttctcaatgtgtaaatttaactactagaactcaattaccaccagcttatactaattcttttactagaggagtatattatccagataaagtatttagatcttctgtattacattctactcaagatttatttttaccattcttctctaatgtaacttggtttcatgctattcatgtatctggaactaatggaactaaaagatttgataatccagtattaccatttaatgatggagtatattttgcttctactgaaaaatctaatattattagaggatggatttttggaactactttagattctaaaactcaatctttattaattgtaaataatgctactaatgtagtaattaaagtatgtgaatttcaattttgtaatgatccatttttaggagtatattatcataaaaataataaatcttggatggaatctgaatttagagtatattcttctgctaataattgtacttttgaatatgtatctcaaccatttttaatggatttagaaggaaaacaaggaaattttaaaaatttaagagaatttgtatttaaaaatattgatggatattttaaaatttattctaaacatactccaattaatttagtaagagatttaccacaaggattttctgctttagaaccattagtagatttaccaattggaattaatattactagatttcaaactttattagctttacatagatcttatttaactccaggagattcttcttctggatggactgctggagctgctgcttattatgtaggatatttacaaccaagaactttcttattaaaatataatgaaaatggaactattactgatgctgtagattgtgctttagatccattatctgaaactaaatgtactttaaaatcttttactgtagaaaaaggaatttatcaaacttctaattttagagtacaaccaactgaatctattgtaagatttccaaatattactaatttatgtccatttggagaagtatttaatgctactagatttgcttctgtatatgcttggaatagaaaaagaatttctaattgtgtagctgattattctgtattatataattctgcttctttctctacttttaaatgttatggagtatctccaactaaattaaatgatttatgttttactaatgtatatgctgattcttttgtaattagaggagatgaagtaagacaaattgctccaggacaaactggaaaaattgctgattataattataaattaccagatgattttactggatgtgtaattgcttggaattctaataatttagattctaaagtaggaggaaattataattatttatatagattatttagaaaatctaatttaaaaccatttgaaagagatatttctactgaaatttatcaagctggatctactccatgtaatggagtagaaggatttaattgttattttccattacaatcttatggatttcaaccaactaatggagtaggatatcaaccatatagagtagtagtattatcttttgaattattacatgctccagctactgtatgtggaccaaaaaaatctactaatttagtaaaaaataaatgtgtaaattttaattttaatggattaactggaactggagtattaactgaatctaataaaaaatttttaccatttcaacaatttggaagagatattgctgatactactgatgctgtaagagatccacaaactttagaaattttagatattactccatgttcttttggaggagtatctgtaattactccaggaactaatacttctaatcaagtagctgtattatatcaaggagtaaattgtactgaagtaccagtagctattcatgctgatcaattaactccaacttggagagtatattctactggatctaatgtatttcaaactagagctggatgtttaattggagctgaacatgtaaataattcttatgaatgtgatattccaattggagctggaatttgtgcttcttatcaaactcaaactaattctccaagaagagctagatctgtagcttctcaatctattattgcttatactatgtctttaggagctgaaaattctgtagcttattctaataattctattgctattccaactaattttactatttctgtaactactgaaattttaccagtatctatgactaaaacttctgtagattgtactatgtatatttgtggagattctactgaatgttctaatttattattacaatatggatctttttgtactcaattaaatagagctttaactggaattgctgtagaacaagataaaaatactcaagaagtatttgctcaagtaaaacaaatttataaaactccaccaattaaagattttggaggatttaatttctctcaaattttaccagatccatctaaaccatctaaaagatcttttattgaagatttattatttaataaagtaactttagctgatgctggatttattaaacaatatggagattgtttaggagatattgctgctagagatttaatttgtgctcaaaaatttaatggattaactgtattaccaccattattaactgatgaaatgattgctcaatatacttctgctttattagctggaactattacttctggatggacttttggagctggagctgctttacaaattccatttgctatgcaaatggcttatagatttaatggaattggagtaactcaaaatgtattatatgaaaatcaaaaattaattgctaatcaatttaattctgctattggaaaaattcaagattctttatcttctactgcttctgctttaggaaaattacaagatgtagtaaatcaaaatgctcaagctttaaatactttagtaaaacaattatcttctaattttggagctatttcttctgtattaaatgatattttatctagattagataaagtagaagctgaagtacaaattgatagattaattactggaagattacaatctttacaaacttatgtaactcaacaattaattagagctgctgaaattagagcttctgctaatttagctgctactaaaatgtctgaatgtgtattaggacaatctaaaagagtagatttttgtggaaaaggatatcatttaatgtcttttccacaatctgctccacatggagtagtatttttacatgtaacttatgtaccagctcaagaaaaaaattttactactgctccagctatttgtcatgatggaaaagctcattttccaagagaaggagtatttgtatctaatggaactcattggtttgtaactcaaagaaatttctatgaaccacaaattattactactgataatacttttgtatctggaaattgtgatgtagtaattggaattgtaaataatactgtatatgatccattacaaccagaattagattcttttaaagaagaattagataaatattttaaaaatcatacttctccagatgtagatttaggagatatttctggaattaatgcttctgtagtaaatattcaaaaagaaattgatagattaaatgaagtagctaaaaatttaaatgaatctttaattgatttacaagaattaggaaaatatgaacaatatattaaatggccatggtatatttggttaggatttattgctggattaattgctattgtaatggtaactattatgttatgttgtatgacttcttgttgttcttgtttaaaaggatgttgttcttgtggatcttgttgtaaatttgatgaagatgattctgaaccagtattaaaaggagtaaaattacattatacttaa

SEQ ID NO: 13 - protein, 1347 aa, Artificial Sequence
  M5 (amino acid sequence)
MIHSVFLLMFLLTPTESYVDVGPDSVKSACIEVDIQQTFFDKTWPRPIDVSKADGIIYPQGRTYSNITITYQGLFPYQGDHGDMYVYSAGHATGTTPQKLFVANYSQDVKQFANGFVVRIGAAANSTGTVIISPSTSATIRKIYPAFMLGSSVGNFSDGKMGRFFNHTLVLLPDGCGTLLRAFYCILEPRSGNHCPAGNSYTSFATYHTPATDCSDGNYNRNASLNSFKEYFNLRNCTFMYTYNITEDEILEWFGITQTAQGVHLFSSRYVDLYGGNMFQFATLPVYDTIKYYSIIPHSIRSIQSDRKAWAAFYVYKLQPLTFLLDFSVDGYIRRAIDCGFNDLSQLHCSYESFDVESGVYSVSSFEAKPSGSVVEQAEGVECDFSPLLSGTPPQVYNFKRLVFTNCNYNLTKLLSLFSVNDFTCSQISPAAIASNCYSSLILDYFSYPLSMKSDLSVSSAGPISQFNYKQSFSNPTCLILATVPHNLTTITKPLKYSYINKCSRLLSDDRTEVPQLVNANQYSPCVSIVPSTVWEDGDYYRKQLSPLEGGGWLVASGSTVAMTEQLQMGFGITVQYGTDTNSVCPKLEFANDTKIASQLGNCVEYSLYGVSGRGVFQNCTAVGVRQQRFVYDAYQNLVGYYSDDGNYYCLRACVSVPVSVIYDKETKTHATLFGSVACEHISSTMSQYSRSTRSMLKRRDSTYGPLQTPVGCVLGLVNSSLFVEDCKLPLGQSLCALPDTPSTLTPRSVRSVPGEMRLASIAFNHPIQVDQLNSSYFKLSIPTNFSFGVTQEYIQTTIQKVTVDCKQYVCNGFQKCEQLLREYGQFCSKINQALHGANLRQDDSVRNLFASVKSSQSSPIIPGFGGDFNLTLLEPVSISTGSRSARSAIEDLLFDKVTIADPGYMQGYDDCMQQGPASARDLICAQKFNGLTVLPPLLTDDMIAAYTAALVSGTATAGWTFGAGAALQIPFAMQMAYRFNGIGVTQNVLYENQKQIANQFNKAISQIQESLTTTSTALGKLQDVVNQNAQALNTLVKQLSSNFGAISSVLNDILSRLDPPEAEVQIDRLITGRLQSLQTYVTQQLIRAAEIRASANLAATKMSECVLGQSKRVDFCGKGYHLMSFPQAAPHGVVFLHVTYVPSQEKNFTTAPAICHEGKAYFPREGVFVFNGTSWFITQRNFFSPQIITTDNTFVSGNCDVVIGIINNTVYDPLQPELDSFKEELDKYFKNHTSPDVDLGDISGINASVVNIQKEIDRLNEVAKNLNESLIDLQELGKYEQYIKWPWYVWLGFIAGLIAIVMVTILLCCMTSCCSCLKGACSCGSCCKFDEDDSEPVLKGVKLHYT

SEQ ID NO: 14 - DNA, 4044 bp, Artificial Sequence
  M5 (nucleic acid sequence)
atgatccattctgtcttcttgcttatgtttttgttgacgcccactgagtcttacgtggacgtgggcccggactctgttaagagcgcatgcattgaggtcgatatacaacaaacattttttgacaagacctggccccggccgatagacgttagcaaagcagatggaataatttatccccaggggcgtacttattccaacataacgatcacataccagggcctgttcccgtatcaaggcgaccacggtgatatgtacgtatacagtgcgggccatgcgacgggcacgacgccgcagaagttgtttgtagccaactacagtcaagatgtcaagcaattcgccaacggcttcgtcgtacgcatcggtgcagctgcgaattctaccggtaccgtgattattagtccgtcgacctcagctaccattcgaaaaatctatccagcgttcatgctcggttcctcagttgggaacttttctgacgggaaaatgggtcggttcttcaatcataccctcgtcctcctcccagatggatgcggcacactgcttcgcgccttctattgcatactagaaccaagatccggcaaccattgccctgcagggaacagctatacatcctttgcaacctatcacactccagcgaccgactgttctgatggtaactataatagaaatgcgtcactaaacagctttaaggagtattttaatttacgcaactgtacctttatgtacacgtataatatcacagaggatgagattctcgagtggttcggtataactcaaacggctcaaggggtgcatttattctcctcacggtatgtcgacctgtacggcggaaatatgttccaattcgccaccttgccggtatacgacactattaagtactactctattatcccacatagcatccgttcaatccagagtgatcgcaaagcttgggctgcgttctatgtgtacaagttgcaacccttaactttcttgctagactttagcgtcgatggttacatccgaagagccattgactgtggattcaacgacctatcgcaactgcattgttcatacgagtcgttcgatgtcgaaagcggtgtttattcagtcagtagctttgaagccaagccgtcgggctctgttgtcgaacaggcggaaggagtagaatgcgacttttccccgctactatcaggcactcctcctcaagtgtacaatttcaaaagactagtattcacaaactgtaattacaaccttaccaaattactatcgctcttttccgtcaacgattttacctgctcacagatttctcctgccgcgatagcatctaattgctactcttctttgattcttgattacttttcgtatccactttccatgaagtctgatttgtcagtatcctctgctggcccgatctcccagtttaattacaagcagtcttttagtaatcccacgtgtctaattcttgctaccgtacctcacaacttaacaacgataacaaagcccctaaagtactcgtacattaacaagtgttccaggttactgtcggatgatcggacggaggttccacaattagtcaacgccaaccaatactcaccatgcgtgtccatagtgccctccacagtatgggaagatggagattactatcggaaacagctatctccattagaaggggggggttggcttgtcgcctcaggatccacagtagctatgactgagcaattacaaatgggttttgggatcacggtgcagtacgggacggacacaaatagtgtatgtccaaagctagagttcgccaatgacaccaaaatcgcctcacagctaggcaattgtgtggaatattctttatatggtgtttcgggccgaggagtattccagaattgtaccgccgttggagttcggcaacagaggttcgtttatgatgcctaccaaaatctggtcggctattattcggatgacggtaactattattgcttaagagcatgcgtttccgtacccgttagcgttatctacgataaggaaacaaaaacccatgcaacactatttggtagcgtagcctgtgaacatatctcgtccaccatgtcgcagtattccaggtctactcgttccatgctgaagcggcgtgactctacatatggaccactgcagactccggtggggtgcgtattgggactcgtcaattctagtctttttgtagaagattgtaaattgcccctgggacaatctttatgcgctctgccagatacaccaagtactttgacaccacgaagtgtgaggtcggtgcccggtgaaatgcgtcttgcatcgattgcgttcaaccaccctatacaagtcgaccaattaaattcctcctattttaaactttcaatcccaactaacttttcttttggggtgacgcaggaatatatccaaaccaccatccaaaaagtcaccgtagattgcaagcagtacgtgtgtaatggttttcaaaaatgcgagcaacttttacgagagtacggtcagttctgttccaaaatcaatcaagctctccacggggcgaacttgaggcaagacgactcggtacgtaatctgtttgcctccgtcaaaagttcgcaatcgtctccgatcatcccgggcttcgggggagactttaatctgacgctgctagaacctgtatcaatttccacgggctcgagaagcgccaggagtgccatagaggacctactgttcgacaaagtaacgatagcagaccctggatacatgcagggttatgatgactgtatgcagcaaggccccgctagcgctcgagacttgatttgcgcacaaaagtttaatggtctcaccgtgcttcccccgctactgactgatgacatgatcgccgcatatacggcagcgttagtatccggaacggcaacagcgggttggacattcggcgcaggcgctgccttacagataccattcgcaatgcagatggcataccgattcaacggtatcggggttacccagaacgtactttatgaaaaccaaaaacaaattgccaaccaattcaataaagcaatttcgcagatccaggagagcttgacaacaacgtcgacggccctcggcaagctacaggacgtggtaaaccagaatgcacaggctcttaatacacttgtaaaacagttatcatcaaattttggcgcgatctcttctgtgctgaatgacatcctgtcgcgtctcgatccacctgaggcggaggtccagatagacaggttgataacgggtcgtttacagtcattgcagacatacgttacacaacaactcattcgagcagcagagatacgcgcgtccgctaacctagcggctaccaaaatgtccgaatgtgtgctaggccaatcgaaacgagtagatttctgtgggaaaggctaccacctcatgtcctttccccaagcagctccacatggcgtggtctttctacatgtcacgtacgtgccttcacaagaaaagaattttaccaccgcgcctgcaatttgccacgaggggaaagcctattttccgagggaaggggttttcgttttcaatgggacctcttggttcattacccaacgtaatttcttctcgccacaaattattactacggacaatactttcgtaagtgggaactgtgatgtagttattggaataatcaacaatacagtctatgaccccctccagccagaactggactctttcaaagaagagcttgataagtatttcaagaatcacaccagccctgacgtggacctaggagatatatcagggataaacgcatcagtggtgaatatacagaaggagattgaccggctaaacgaagtcgcgaagaaccttaacgagtcgttaattgacctgcaagaactcgggaagtacgaacagtacattaagtggccttggtacgtatggttagggtttatagccggactcatcgcgatagtcatggtgactattctcctctgctgcatgacatcttgctgcagctgtctgaagggggcatgtagttgtggcagctgttgcaaatttgacgaggatgatagcgaaccggtgcttaagggcgtaaaattacactacacctaa

SEQ ID NO: 15 - protein, 1347 aa, Artificial Sequence
  M5 + D510G (amino acid sequence)
MIHSVFLLMFLLTPTESYVDVGPDSVKSACIEVDIQQTFFDKTWPRPIDVSKADGIIYPQGRTYSNITITYQGLFPYQGDHGDMYVYSAGHATGTTPQKLFVANYSQDVKQFANGFVVRIGAAANSTGTVIISPSTSATIRKIYPAFMLGSSVGNFSDGKMGRFFNHTLVLLPDGCGTLLRAFYCILEPRSGNHCPAGNSYTSFATYHTPATDCSDGNYNRNASLNSFKEYFNLRNCTFMYTYNITEDEILEWFGITQTAQGVHLFSSRYVDLYGGNMFQFATLPVYDTIKYYSIIPHSIRSIQSDRKAWAAFYVYKLQPLTFLLDFSVDGYIRRAIDCGFNDLSQLHCSYESFDVESGVYSVSSFEAKPSGSVVEQAEGVECDFSPLLSGTPPQVYNFKRLVFTNCNYNLTKLLSLFSVNDFTCSQISPAAIASNCYSSLILDYFSYPLSMKSDLSVSSAGPISQFNYKQSFSNPTCLILATVPHNLTTITKPLKYSYINKCSRLLSDGRTEVPQLVNANQYSPCVSIVPSTVWEDGDYYRKQLSPLEGGGWLVASGSTVAMTEQLQMGFGITVQYGTDTNSVCPKLEFANDTKIASQLGNCVEYSLYGVSGRGVFQNCTAVGVRQQRFVYDAYQNLVGYYSDDGNYYCLRACVSVPVSVIYDKETKTHATLFGSVACEHISSTMSQYSRSTRSMLKRRDSTYGPLQTPVGCVLGLVNSSLFVEDCKLPLGQSLCALPDTPSTLTPRSVRSVPGEMRLASIAFNHPIQVDQLNSSYFKLSIPTNFSFGVTQEYIQTTIQKVTVDCKQYVCNGFQKCEQLLREYGQFCSKINQALHGANLRQDDSVRNLFASVKSSQSSPIIPGFGGDFNLTLLEPVSISTGSRSARSAIEDLLFDKVTIADPGYMQGYDDCMQQGPASARDLICAQKFNGLTVLPPLLTDDMIAAYTAALVSGTATAGWTFGAGAALQIPFAMQMAYRFNGIGVTQNVLYENQKQIANQFNKAISQIQESLTTTSTALGKLQDVVNQNAQALNTLVKQLSSNFGAISSVLNDILSRLDPPEAEVQIDRLITGRLQSLQTYVTQQLIRAAEIRASANLAATKMSECVLGQSKRVDFCGKGYHLMSFPQAAPHGVVFLHVTYVPSQEKNFTTAPAICHEGKAYFPREGVFVFNGTSWFITQRNFFSPQIITTDNTFVSGNCDVVIGIINNTVYDPLQPELDSFKEELDKYFKNHTSPDVDLGDISGINASVVNIQKEIDRLNEVAKNLNESLIDLQELGKYEQYIKWPWYVWLGFIAGLIAIVMVTILLCCMTSCCSCLKGACSCGSCCKFDEDDSEPVLKGVKLHYT

SEQ ID NO: 16 - protein, 1347 aa, Artificial Sequence
  M5 + I529T (amino acid sequence)
MIHSVFLLMFLLTPTESYVDVGPDSVKSACIEVDIQQTFFDKTWPRPIDVSKADGIIYPQGRTYSNITITYQGLFPYQGDHGDMYVYSAGHATGTTPQKLFVANYSQDVKQFANGFVVRIGAAANSTGTVIISPSTSATIRKIYPAFMLGSSVGNFSDGKMGRFFNHTLVLLPDGCGTLLRAFYCILEPRSGNHCPAGNSYTSFATYHTPATDCSDGNYNRNASLNSFKEYFNLRNCTFMYTYNITEDEILEWFGITQTAQGVHLFSSRYVDLYGGNMFQFATLPVYDTIKYYSIIPHSIRSIQSDRKAWAAFYVYKLQPLTFLLDFSVDGYIRRAIDCGFNDLSQLHCSYESFDVESGVYSVSSFEAKPSGSVVEQAEGVECDFSPLLSGTPPQVYNFKRLVFTNCNYNLTKLLSLFSVNDFTCSQISPAAIASNCYSSLILDYFSYPLSMKSDLSVSSAGPISQFNYKQSFSNPTCLILATVPHNLTTITKPLKYSYINKCSRLLSDDRTEVPQLVNANQYSPCVSTVPSTVWEDGDYYRKQLSPLEGGGWLVASGSTVAMTEQLQMGFGITVQYGTDTNSVCPKLEFANDTKIASQLGNCVEYSLYGVSGRGVFQNCTAVGVRQQRFVYDAYQNLVGYYSDDGNYYCLRACVSVPVSVIYDKETKTHATLFGSVACEHISSTMSQYSRSTRSMLKRRDSTYGPLQTPVGCVLGLVNSSLFVEDCKLPLGQSLCALPDTPSTLTPRSVRSVPGEMRLASIAFNHPIQVDQLNSSYFKLSIPTNFSFGVTQEYIQTTIQKVTVDCKQYVCNGFQKCEQLLREYGQFCSKINQALHGANLRQDDSVRNLFASVKSSQSSPIIPGFGGDFNLTLLEPVSISTGSRSARSAIEDLLFDKVTIADPGYMQGYDDCMQQGPASARDLICAQKFNGLTVLPPLLTDDMIAAYTAALVSGTATAGWTFGAGAALQIPFAMQMAYRFNGIGVTQNVLYENQKQIANQFNKAISQIQESLTTTSTALGKLQDVVNQNAQALNTLVKQLSSNFGAISSVLNDILSRLDPPEAEVQIDRLITGRLQSLQTYVTQQLIRAAEIRASANLAATKMSECVLGQSKRVDFCGKGYHLMSFPQAAPHGVVFLHVTYVPSQEKNFTTAPAICHEGKAYFPREGVFVFNGTSWFITQRNFFSPQIITTDNTFVSGNCDVVIGIINNTVYDPLQPELDSFKEELDKYFKNHTSPDVDLGDISGINASVVNIQKEIDRLNEVAKNLNESLIDLQELGKYEQYIKWPWYVWLGFIAGLIAIVMVTILLCCMTSCCSCLKGACSCGSCCKFDEDDSEPVLKGVKLHYT

SEQ ID NO: 17 - protein, 1347 aa, Artificial Sequence
  M5 + D510G + I529T (amino acid sequence)
MIHSVFLLMFLLTPTESYVDVGPDSVKSACIEVDIQQTFFDKTWPRPIDVSKADGIIYPQGRTYSNITITYQGLFPYQGDHGDMYVYSAGHATGTTPQKLFVANYSQDVKQFANGFVVRIGAAANSTGTVIISPSTSATIRKIYPAFMLGSSVGNFSDGKMGRFFNHTLVLLPDGCGTLLRAFYCILEPRSGNHCPAGNSYTSFATYHTPATDCSDGNYNRNASLNSFKEYFNLRNCTFMYTYNITEDEILEWFGITQTAQGVHLFSSRYVDLYGGNMFQFATLPVYDTIKYYSIIPHSIRSIQSDRKAWAAFYVYKLQPLTFLLDFSVDGYIRRAIDCGFNDLSQLHCSYESFDVESGVYSVSSFEAKPSGSVVEQAEGVECDFSPLLSGTPPQVYNFKRLVFTNCNYNLTKLLSLFSVNDFTCSQISPAAIASNCYSSLILDYFSYPLSMKSDLSVSSAGPISQFNYKQSFSNPTCLILATVPHNLTTITKPLKYSYINKCSRLLSDGRTEVPQLVNANQYSPCVSTVPSTVWEDGDYYRKQLSPLEGGGWLVASGSTVAMTEQLQMGFGITVQYGTDTNSVCPKLEFANDTKIASQLGNCVEYSLYGVSGRGVFQNCTAVGVRQQRFVYDAYQNLVGYYSDDGNYYCLRACVSVPVSVIYDKETKTHATLFGSVACEHISSTMSQYSRSTRSMLKRRDSTYGPLQTPVGCVLGLVNSSLFVEDCKLPLGQSLCALPDTPSTLTPRSVRSVPGEMRLASIAFNHPIQVDQLNSSYFKLSIPTNFSFGVTQEYIQTTIQKVTVDCKQYVCNGFQKCEQLLREYGQFCSKINQALHGANLRQDDSVRNLFASVKSSQSSPIIPGFGGDFNLTLLEPVSISTGSRSARSAIEDLLFDKVTIADPGYMQGYDDCMQQGPASARDLICAQKFNGLTVLPPLLTDDMIAAYTAALVSGTATAGWTFGAGAALQIPFAMQMAYRFNGIGVTQNVLYENQKQIANQFNKAISQIQESLTTTSTALGKLQDVVNQNAQALNTLVKQLSSNFGAISSVLNDILSRLDPPEAEVQIDRLITGRLQSLQTYVTQQLIRAAEIRASANLAATKMSECVLGQSKRVDFCGKGYHLMSFPQAAPHGVVFLHVTYVPSQEKNFTTAPAICHEGKAYFPREGVFVFNGTSWFITQRNFFSPQIITTDNTFVSGNCDVVIGIINNTVYDPLQPELDSFKEELDKYFKNHTSPDVDLGDISGINASVVNIQKEIDRLNEVAKNLNESLIDLQELGKYEQYIKWPWYVWLGFIAGLIAIVMVTILLCCMTSCCSCLKGACSCGSCCKFDEDDSEPVLKGVKLHYT

SEQ ID NO: 18 - protein, 1347 aa, Artificial Sequence
  Mosaic MERS-CoV/Bat SARS-like CoV S Protein
MIHSVFLLMFLLTPTESYVDVGPDSVKSACIEVDIQQTFFDKTWPRPIDVSKADGIIYPQGRTYSNITITYQGLFPYQGDHGDMYVYSAGHATGTTPQKLFVANYSQDVKQFANGFVVRIGAAANSTGTVIISPSTSATIRKIYPAFMLGSSVGNFSDGKMGRFFNHTLVLLPDGCGTLLRAFYCILEPRSGNHCPAGNSYTSFATYHTPATDCSDGNYNRNASLNSFKEYFNLRNCTFMYTYNITEDEILEWFGITQTAQGVHLFSSRYVDLYGGNMFQFATLPVYDTIKYYSIIPHSIRSIQSDRKAWAAFYVYKLQPLTFLLDFSVDGYIRRAIDCGFNDLSQLHCSYESFDVESGVYSVSSFEAKPSGSVVEQAEGVECDFSPLLSGTPPQVYNFKRLVFTNCNYNLTKLLSLFSVNDFTCSQISPAAIASNCYSSLILDYFSYPLSMKSDLSVSSAGPISQFNYKQSFSNPTCLILATVPHNLTTITKPLKYSYINKCSRLLSDDRTEVPQLVNANQYSPCVSIVPSTVWEDGDYYRKQLSPLEGGGWLVASGSTVAMTEQLQMGFGITVQYGTDTNSVCPKLEFANDTKIASQLGNCVEYSLYGVSGRGVFQNCTAVGVRQQRFVYDAYQNLVGYYSDDGNYYCLRACVSVPVSVIYDKETKTHATLFGSVACEHISSTMSQYSRSTRSMLKRRDSTYGPLQTPVGCVLGLVNSSLFVEDCKLPLGQSLCALPDTPSTLTPRSVRSVPGEMRLASIAFNHPIQVDQLNSSYFKLSIPTNFSFGVTQEYIQTTIQKVTVDCKQYVCNGFQKCEQLLREYGQFCSKINQALHGANLRQDDSVRNLFASVKSSQSSPIIPGFGGDFNLTLLEPVSISTGSRSARSAIEDLLFDKVTIADPGYMQGYDDCMQQGPASARDLICAQKFNGLTVLPPLLTDDMIAAYTAALVSGTATAGWTFGAGAALQIPFAMQMAYRFNGIGVTQNVLYENQKQIANQFNKAISQIQESLTTTSTALGKLQDVVNQNAQALNTLVKQLSSNFGAISSVLNDILSRLDKVEAEVQIDRLITGRLQSLQTYVTQQLIRAAEIRASANLAATKMSECVLGQSKRVDFCGKGYHLMSFPQAAPHGVVFLHVTYVPSQEKNFTTAPAICHEGKAYFPREGVFVFNGTSWFITQRNFFSPQIITTDNTFVSGNCDVVIGIINNTVYDPLQPELDSFKEELDKYFKNHTSPDVDLGDISGINASVVNIQKEIDRLNEVAKNLNESLIDLQELGKYEQYIKWPWYVWLGFIAGLIAIVMVTILLCCMTSCCSCLKGACSCGSCCKFDEDDSEPVLKGVKLHYT